European Patent Application EP 4 756 023 A1, published June 10, 2026. Title: Self-cleavable ribozyme therapeutic nucleic acid molecules. Applicant: Max-Planck-Gesellschaft zur Förderung der Wissenschaften e.V. The sequence listing filed with the application follows.

SEQUENCE LISTING (6 sequences)

SEQ ID NO: 1 - DNA, 12 bp, synthetic construct
  source 1..12: mol_type = other DNA; note = insulator sequence
caaacaaacaaa

SEQ ID NO: 2 - DNA, 10 bp, synthetic construct
  source 1..10: mol_type = other DNA; note = Kozak sequence
gccaccatgg

SEQ ID NO: 3 - skipped

SEQ ID NO: 4 - DNA, 1320 bp, synthetic construct
  source 1..1320: mol_type = other DNA; note = DMD exons E29 to E34
tcacttgaaaatttgatgcgacattcagaggataacccaaatcagattcgcatattggcacagaccctaacagatggcggagtcatggatgagctaatcaatgaggaacttgagacatttaattctcgttggagggaactacatgaagaggctgtaaggaggcaaaagttgcttgaacagagcatccagtctgcccaggagactgaaaaatccttacacttaatccaggagtccctcacattcattgacaagcagttggcagcttatattgcagacaaggtggacgcagctcaaatgcctcaggaagcccagaaaatccaatctgatttgacaagtcatgagatcagtttagaagaaatgaagaaacataatcaggggaaggaggctgcccaaagagtcctgtctcagattgatgttgcacaggtatatgttatttcagaaactaaggaacgtgttttcgttgggcattatactccagtctatattggacaacttgattattggcaagattggatttgaggacattatttgaaaactataatttgatgtctaaacaatgagtgttttgctctctacattttaaagataaaataggttaataaattaccttttatttagtataacattaagaaaaaactactgaatcattctcccaaatgtatgttttcctgtgttggatgaatggaaaaatactgctttattttgtttttatttttctgtatatcttcagaaataaaggcagatctatcaataaaaataggaccagttattgtttgaaaggcaaaattaaatcagtgcctttttacactgtccttacagaaaaaattacaagatgtctccatgaagtttcgattattccagaaaccagccaattttgagcagcgtctacaagaaagtaagatgattttagatgaagtgaagatgcacttgcctgcattggaaacaaagagtgtggaacaggaagtagtacagtcacagctaaatcattgtgtgaacttgtataaaagtctgagtgaagtgaagtctgaagtggaaatggtgataaagactggacgtcagattgtacagaaaaagcagacggaaaatcccaaagaacttgatgaaagagtaacagctttgaaattgcattataatgagctgggagcaaaggtaacagaaagaaagcaacagttggagaaatgcttgaaattgtcccgtaagatgcgaaaggaaatgaatgtcttgacagaatggctggcagctacagatatggaattgacaaagagatcagcagttgaaggaatgcctagtaatttggattctgaagttgcctggggaaag

SEQ ID NO: 5 - DNA, 1689 bp, synthetic construct
  source 1..1689: mol_type = other DNA; note = DMD RIBOZYME MINIGENE SEQUENCE
gccaccatggattcacttgaaaatttgatgcgacattcagaggataacccaaatcagattcgcatattggcacagaccctaacagatggcggagtcatggatgagctaatcaatgaggaacttgagacatttaattctcgttggagggaactacatgaagaggctgtaaggaggcaaaagttgcttgaacagagcatccagtctgcccaggagactgaaaaatccttacacttaatccaggagtccctcacattcattgacaagcagttggcagcttatattgcagacaaggtggacgcagctcaaatgcctcaggaagcccagaaaatccaatctgatttgacaagtcatgagatcagtttagaagaaatgaagaaacataatcaggggaaggaggctgcccaaagagtcctgtctcagattgatgttgcacaggtatatgttatttcagaaactaaggaacgtgttttcgttgggcattatactccagtctatattcaaacaaacaaagcgcgtcctggattccacttcgggtacatccagctgacgagtcccaaataggacgaaacgcgccaaacaaacaaaggacaacttgattattggcaagattggatttgaggacattatttgaaaactataatttgatgtctaaacaatgagtgttttgctctctacattttaaagataaaataggttaataaattaccttttatttagtataacattaagaaaaaactactgaatcattctcccaaatgtatgttttcctgtgttggatgaatggaaaaatactgctttattttgtttttatttttctgtatatcttcagaaataaaggcagatctatcaataaaaataggaccagttattgtttgaaaggcaaaattaaatcagtgcctttttacactgtccttacagaaaaaattacaagatgtctccatgaagtttcgattattccagaaaccagccaattttgagcagcgtctacaagaaagtaagatgattttagatgaagtgaagatgcacttgcctgcattggaaacaaagagtgtggaacaggaagtagtacagtcacagctaaatcattgtgtgaacttgtataaaagtctgagtgaagtgaagtctgaagtggaaatggtgataaagactggacgtcagattgtacagaaaaagcagacggaaaatcccaaagaacttgatgaaagagtaacagctttgaaattgcattataatgagctgggagcaaaggtaacagaaagaaagcaacagttggagaaatgcttgaaattgtcccgtaagatgcgaaaggaaatgaatgtcttgacagaatggctggcagctacagatatggaattgacaaagagatcagcagttgaaggaatgcctagtaatttggattctgaagttgcctggggaaagccaagcttggggatcaattctctagagctcgctgatcagcctcgactgtgccttctagttgccagccatctgttgtttgcccctcccccgtgccttccttgaccctggaaggtgccactcccactgtcctttcctaataaaatgaggaaattgcatcgcattgtctgagtaggtgtcattctattctggggggtggggtggggcaggacagcaagggggaggattgggaagacaatagcaggcatgctggggatgcggtgggctctatgg

SEQ ID NO: 6 - DNA, 63 bp, synthetic construct
  source 1..63: mol_type = other DNA; note = self-cleavable ribozyme
gcgcgtcctggattccacttcgggtacatccagctgacgagtcccaaataggacgaaacgcgc